European Patent Application EP 4 410 955 A1, published August 7, 2024. Title: METHOD FOR CULTURING MICROORGANISM, TRANSFORMED MICROORGANISM, AND METHOD FOR PRODUCING POLY(3-HYDROXYALKANOATE). Applicant: Kaneka Corporation. Application EP 22 876 375.1, filed September 28, 2022. The sequence listing filed with the application follows.

SEQUENCE LISTING (2 sequences)

SEQ ID NO: 1 - protein, 672 aa, Escherichia coli
MSYPSLFAPLDLGFTTLKNRVLMGSMHTGLEEYPDGAERLAAFYAERARHGVALIVSGGIAPDLTGVGMEGGAMLNDASQIPHHRTITEAVHQEGGKIALQILHTGRYSYQPHLVAPSALQAPINRFVPHELSHEEILQLIDNFARCAQLAREAGYDGVEVMGSEGYLINEFLTLRTNQRSDQWGGDYRNRMRFAVEVVRAVRERVGNDFIIIYRLSMLDLVEDGGTFAETVELAQAIEAAGATIINTGIGWHEARIPTIATPVPRGAFSWVTRKLKGHVSLPLVTTNRINDPQVADDILSRGDADMVSMARPFLADAELLSKAQSGRADEINTCIGCNQACLDQIFVGKVTSCLVNPRACHETKMPILPAVQKKNLAVVGAGPAGLAFAINAAARGHQVTLFDAHSEIGGQFNIAKQIPGKEEFYETLRYYRRMIEVTGVTLKLNHTVTADQLQAFDETILASGIVPRTPPIDGIDHPKVLSYLDVLRDKAPVGNKVAIIGCGGIGFDTAMYLSQPGESTSQNIAGFCNEWGIDSSLQQAGGLSPQGMQIPRSPRQIVMLQRKASKPGQGLGKTTGWIHRTTLLSRGVKMIPGVSYQKIDDDGLHVVINGETQVLAVDNVVICAGQEPNRALAQPLIDSGKTVHLIGGCDVAMELDARRAIAQGTRLALEI

SEQ ID NO: 2 - DNA, 2319 bp, synthetic construct
  source 1..2319: mol_type = other DNA
gaattctgcttctggcgtcaggcagccatcggaagctgtggtatggctgtgcaggtcgtaaatcactgcataattcgtgtcgctcaaggcgcactcccgttctggataatgttttttgcgccgacatcataacggttctggcaaatattctgaaatgagctgttgacaattaatcatcgaactagttaactagtacgcaagttcacagcggataacaatttcacacaggaaacaattccacgtgcagagagacaatcaaatcatgagctacccgtcgctgttcgccccgctggatttaggttttaccacgttaaaaaaccgcgtgttgatgggctcaatgcacaccgggctggaggaatacccggacggtgccgagcggctggcagcgttttatgccgaacgcgcccgtcacggcgtggcgctgattgtcagcggcggcattgcaccagatttaacaggcgttggcatggaaggtggcgcaatgctcaacgacgccagccagatcccacaccatcgcaccattaccgaagcggtacatcaggaaggcggcaaaatagccctgcaaattttgcataccgggcgctacagctaccaaccgcatctggtcgccccgtccgcattgcaggcccccatcaaccgtttcgtgccccatgagttaagccatgaagagatcctgcaactgatcgacaatttcgcccgctgcgcgcaactggcgcgggaggcaggatacgacggtgtagaggtgatgggttccgaagggtatttgatcaacgaatttctgacgctgcgcaccaatcagcgtagtgaccagtggggcggcgattaccgcaaccggatgcgatttgccgtagaagtagtgcgtgcggtgcgcgaacgcgtcggcaacgacttcattattatctaccgactgtcgatgctcgacctggtcgaagacggcgggacttttgccgaaacggtagagctggcgcaggccattgaagcggcgggcgcgaccattatcaacaccggcattggctggcatgaagcacgtattccgaccattgccacgcccgtgccgcgcggcgcatttagctgggtcacgcgcaaactgaaaggccacgtctcgctgccgctggtaaccaccaaccggattaacgatccgcaggttgccgacgatattctctcgcgcggcgatgccgatatggtatcgatggcgcgaccgtttcttgctgatgcggagctgctgtcaaaagcgcaatcgggacgagccgatgagatcaacacttgtattggctgcaatcaggcctgtctcgatcaaatcttcgttggcaaagtcacctcgtgcctggtgaatcctcgcgcctgccacgaaaccaaaatgccaatccttcccgccgtgcagaaaaaaaatctggcggtggtcggtgcgggacctgctgggctggcgtttgccattaacgcggcggcgcgtgggcatcaggtaacattgtttgacgctcatagcgagattggcgggcagtttaatatcgccaaacagatccccggcaaagaggagttttacgaaacgctgcgctattaccgccggatgatcgaagtgacgggcgtgacgctaaaactcaatcacaccgtgacggcggatcagttacaggctttcgatgaaacgatcctcgccagtgggatcgtgccgcgcactccgcccatcgacgggatcgatcatccgaaggtattgagttatctcgatgtactgcgcgacaaagcgccggttggcaacaaagttgccatcatcggttgtggcgggattggttttgatacggcgatgtatttaagtcagccgggcgaatccaccagccagaatatcgccgggttctgtaatgaatgggggatcgacagtagcctacaacaggctggtggcttaagcccgcagggaatgcagatcccccgtagcccacggcagattgtgatgctccagcgcaaagccagcaaaccaggacaggggttaggcaaaaccaccggctggatccatcgcaccaccctgctctcgcggggtgtgaaaatgatcccaggcgtaagttatcagaagattgacgatgacgggctgcatgtggtgatcaacggcgaaacgcaggtattagcagtggacaatgtggtgatctgcgcagggcaagagccaaaccgcgcgctggcgcaaccgctgattgatagcgggaaaacggtgcatttaattggcggctgcgatgtggctatggagctggacgcacgacgggcaattgcccagggaacacggctggcgctggagatttaacctgccggcctggttcaaccagtcggcagccgactagt